European Patent Application EP 4 585 616 A1, published July 16, 2025. Title: 能够特异性结合ROR1的抗体、其偶联药物及其制备方法和应用. Applicant: 中国科学院合肥物质科学研究院. Application WO. The sequence listing filed with the application follows.

SEQUENCE LISTING (101 sequences)

SEQ ID NO: 1 - protein, 5 aa, synthetic construct
DYNLH

SEQ ID NO: 2 - protein, 17 aa, synthetic construct
YINPNHDGTSYNQKFQG

SEQ ID NO: 3 - protein, 10 aa, synthetic construct
RVRTGTGLDD

SEQ ID NO: 4 - protein, 16 aa, synthetic construct
RSSHNIVHTNGNTYLE

SEQ ID NO: 5 - protein, 7 aa, synthetic construct
KVSNRFS

SEQ ID NO: 6 - protein, 9 aa, synthetic construct
FQGSRFPYT

SEQ ID NO: 7 - protein, 119 aa, synthetic construct
EVRLQQSGPVLVKPGASVKMSCKASGYTFTDYNLHWVKQSHRQSLEWIGYINPNHDGTSYNQKFQGKATLTVDRSSSTAYMEFRSLTSEDSAVYYCARRVRTGTGLDDWGQGTTLTVSS

SEQ ID NO: 8 - protein, 119 aa, synthetic construct
EVRLQQSGPVLVKPGASVKMSCKASGYTFTDYNLHWVKQSHRQSLEWIGYINPNHDATSYNQKFQGKATLTVDRSSSTAYMEFRSLTSEDSAVYYCARRVRTGTGLDDWGQGTTLTVSS

SEQ ID NO: 9 - protein, 112 aa, synthetic construct
DVLMTQSPLSLPVSLGDQASISCRSSHNIVHTNGNTYLEWYLQKPGQSPKLLIYKVSNRFSGVPDRFSGSGSGTYFTLTISRVEAEDLGVYYCFQGSRFPYTFGGGTKLEIK

SEQ ID NO: 10 - protein, 112 aa, synthetic construct
DVLMTQSPLSLPVSLGDQASISCRSSHNIVHTNANTYLEWYLQKPGQSPKLLIYKVSNRFSGVPDRFSGSGSGTYFTLTISRVEAEDLGVYYCFQGSRFPYTFGGGTKLEIK

SEQ ID NO: 11 - protein, 5 aa, synthetic construct
TYAMH

SEQ ID NO: 12 - protein, 19 aa, synthetic construct
RIRSKSSNFATYYADSVRD

SEQ ID NO: 13 - protein, 11 aa, synthetic construct
GYGPSYFSLDY

SEQ ID NO: 14 - protein, 16 aa, synthetic construct
RSSQSLVHSNGNTYLH

SEQ ID NO: 15 - protein, 7 aa, synthetic construct
KVSNRFS

SEQ ID NO: 16 - protein, 9 aa, synthetic construct
SQSTHAIYT

SEQ ID NO: 17 - protein, 122 aa, synthetic construct
EVQLVESGGGLVQPKGSLKLSCAASGFTFNTYAMHWVRQAPGKGLEWVARIRSKSSNFATYYADSVRDRFTISRDDSQSMLYLQMNNLKTEDTAMYYCVRGYGPSYFSLDYWGQGTSVTVSS

SEQ ID NO: 18 - protein, 112 aa, synthetic construct
DVVMTQTPLSLPVSLGDQASISCRSSQSLVHSNGNTYLHWYLQKPGQSPKLLIYKVSNRFSGVPDRFSGSGSGTDFTLKINRVEAEDLGVYFCSQSTHAIYTFGGGTKLEIK

SEQ ID NO: 19 - protein, 5 aa, synthetic construct
SYAMS

SEQ ID NO: 20 - protein, 17 aa, synthetic construct
TISDGGSYTYYPDNEKG

SEQ ID NO: 21 - protein, 12 aa, synthetic construct
GGYYYNLYAMDY

SEQ ID NO: 22 - protein, 15 aa, synthetic construct
KASQSVSFPGTSLMH

SEQ ID NO: 23 - protein, 7 aa, synthetic construct
RASNLEA

SEQ ID NO: 24 - protein, 9 aa, synthetic construct
QQSREYPWT

SEQ ID NO: 25 - protein, 121 aa, synthetic construct
EVQLVESGGGLVKPGGSLKLSCAASGFTFNSYAMSWVRQTPEKRLEWVATISDGGSYTYYPDNEKGRFTISRDNAKNNLYLQMSHLKSEDTAIYYCVRGGYYYNLYAMDYWGQGTSVTVSS

SEQ ID NO: 26 - protein, 121 aa, synthetic construct
EVQLVESGGGLVKPGGSLKLSCAASGFTFNSYAMSWVRQTPEKRLEWVATISDAGSYTYYPDNEKGRFTISRDNAKNNLYLQMSHLKSEDTAIYYCVRGGYYYNLYAMDYWGQGTSVTVSS

SEQ ID NO: 27 - protein, 111 aa, synthetic construct
DIVLTQSPASLAVSLGQRAIISCKASQSVSFPGTSLMHWYQQKPGQQPKLLIYRASNLEAGVPTRFSGSGSRTDFTLNIHPVEEDDTATYYCQQSREYPWTFGGGTQLEIK

SEQ ID NO: 28 - protein, 119 aa, synthetic construct
QVQLVQSGAEVKKPGASVKVSCKASGYTFTDYNLHWVRQAPGQGLEWMGYINPNHDATSYNQKFQGRVTMTRDTSTSTVYMELSSLRSEDTAVYYCARRVRTGTGLDDWGQGTTVTVSS

SEQ ID NO: 29 - protein, 119 aa, synthetic construct
QVQLVQSGAEVKKPGASVKVSCKASGYTFTDYNLHWVRQAPGQGLEWMGYINPNHDATSYNQKFQGKVTMTVDTSTSTVYMELSSLRSEDTAVYYCARRVRTGTGLDDWGQGTTVTVSS

SEQ ID NO: 30 - protein, 119 aa, synthetic construct
QVQLVQSGAEVKKPGASVKVSCKASGYTFTDYNLHWVKQAPGQGLEWIGYINPNHDATSYNQKFQGKVTMTVDTSTSTVYMELSSLRSEDTAVYYCARRVRTGTGLDDWGQGTTVTVSS

SEQ ID NO: 31 - protein, 119 aa, synthetic construct
QVQLVQSGAEVKKPGASVKVSCKASGYTFTDYNLHWVKQAPGQGLEWIGYINPNHDATSYNQKFQGKATLTVDTSTSTVYMELSSLRSEDTAVYYCARRVRTGTGLDDWGQGTTVTVSS

SEQ ID NO: 32 - protein, 119 aa, synthetic construct
QVQLVQSGAEVKKPGASVKVSCKASGYTFTDYNLHWVKQAPGQGLEWIGYINPNHDATSYNQKFQGKATLTVDTSTSTAYMELSSLTSEDTAVYYCARRVRTGTGLDDWGQGTTVTVSS

SEQ ID NO: 33 - protein, 112 aa, synthetic construct
DVVMTQSPLSLPVTLGQPASISCRSSHNIVHTNANTYLEWYQQRPGQSPRLLIYKVSNRFSGVPDRFSGSGSGTDFTLKISRVEAEDVGVYYCFQGSRFPYTFGGGTKVEIK

SEQ ID NO: 34 - protein, 112 aa, synthetic construct
DVVMTQSPLSLPVTLGQPASISCRSSHNIVHTNANTYLEWYQQRPGQSPKLLIYKVSNRFSGVPDRFSGSGSGTDFTLKISRVEAEDVGVYYCFQGSRFPYTFGGGTKVEIK

SEQ ID NO: 35 - protein, 5 aa, synthetic construct
DYNLH

SEQ ID NO: 36 - protein, 17 aa, synthetic construct
YINPNNGGTTYNQKFKG

SEQ ID NO: 37 - protein, 10 aa, synthetic construct
RVRTGTGFDY

SEQ ID NO: 38 - protein, 16 aa, synthetic construct
KSSHNILHTNGNTYLE

SEQ ID NO: 39 - protein, 7 aa, synthetic construct
KVSNRFS

SEQ ID NO: 40 - protein, 9 aa, synthetic construct
FQGSRFPYT

SEQ ID NO: 41 - protein, 119 aa, synthetic construct
EVQLQQSGPELVKPGASVKMSCKTSGYTFTDYNLHWVKQSHRRSLEWIGYINPNNGGTTYNQKFKGKATLTVDKSSSTAYMELRSLTSEDSAVYYFVRRVRTGTGFDYWGQGTTLTVSS

SEQ ID NO: 42 - protein, 112 aa, synthetic construct
EVLMTQTPLSLPVSLGDQASISCKSSHNILHTNGNTYLEWYLQKPGQSPKLLIYKVSNRFSGVPDRFSGSGSGTDFTLTISRVEAEDLGVYYCFQGSRFPYTFGGGTKLEIK

SEQ ID NO: 43 - protein, 5 aa, synthetic construct
SYAMS

SEQ ID NO: 44 - protein, 17 aa, synthetic construct
TISDGGSYTYYPDSVKG

SEQ ID NO: 45 - protein, 12 aa, synthetic construct
GGYYYNLYAMDY

SEQ ID NO: 46 - protein, 15 aa, synthetic construct
KASQSVSFAGTSLMH

SEQ ID NO: 47 - protein, 7 aa, synthetic construct
RASNLEA

SEQ ID NO: 48 - protein, 9 aa, synthetic construct
QQSGEYPWT

SEQ ID NO: 49 - protein, 121 aa, synthetic construct
EVQLVESGGGLVKPGGSLKLSCAASGFTFSSYAMSWVRQTPEKRLEWVATISDGGSYTYYPDSVKGRFTISRDNAKNNLYLQMSHLKSEDTDMYYCVRGGYYYNLYAMDYWGQGTSVTVSS

SEQ ID NO: 50 - protein, 111 aa, synthetic construct
DIVLTQSPASLAVSLGQRAIISCKASQSVSFAGTSLMHWYQQKPGQQPKLLIYRASNLEAGVPTRFSGSGSRADFTLNIHPVEEDDAATYYCQQSGEYPWTFGGGTKLEIK

SEQ ID NO: 51 - protein, 5 aa, synthetic construct
DYNIH

SEQ ID NO: 52 - protein, 17 aa, synthetic construct
YINPNNGGTTYNQKFKG

SEQ ID NO: 53 - protein, 11 aa, synthetic construct
RGYGSSYAMDY

SEQ ID NO: 54 - protein, 16 aa, synthetic construct
RSSHIIVHTNGNTYLE

SEQ ID NO: 55 - protein, 7 aa, synthetic construct
KVSNRFS

SEQ ID NO: 56 - protein, 9 aa, synthetic construct
FQGSRVPYT

SEQ ID NO: 57 - protein, 120 aa, synthetic construct
EVQLQQSGPELVKPGASLKMSCKASGYTFPDYNIHWVKQSHGKSLEWIGYINPNNGGTTYNQKFKGKATLTVSKSSSTAYMELRSLTSEDSAVYSCARRGYGSSYAMDYWAQGTSVTVSS

SEQ ID NO: 58 - protein, 112 aa, synthetic construct
DVLMTQSPLSLPVSLGDQASISCRSSHIIVHTNGNTYLEWYLQKPGQSPKLLIYKVSNRFSGVPDRFSGSGSGTDFTLKISRVEAEDLGVYYCFQGSRVPYTFGGGTKLEIK

SEQ ID NO: 59 - protein, 5 aa, synthetic construct
DYNMH

SEQ ID NO: 60 - protein, 17 aa, synthetic construct
YINPNNGGTSYNQKFKG

SEQ ID NO: 61 - protein, 11 aa, synthetic construct
RGYGSGYAMDY

SEQ ID NO: 62 - protein, 16 aa, synthetic construct
RSSQSIVHTNGNTYLE

SEQ ID NO: 63 - protein, 7 aa, synthetic construct
KVFNRFS

SEQ ID NO: 64 - protein, 9 aa, synthetic construct
FQGSLFPYT

SEQ ID NO: 65 - protein, 120 aa, synthetic construct
EVQLQQSGPELVKPGASVKMSCKASGYTFTDYNMHWVKQSHGKSLEWIGYINPNNGGTSYNQKFKGKATLTVNKSSSTAYMELRSLTSDDSAVYYCARRGYGSGYAMDYWGQGTSVTVSS

SEQ ID NO: 66 - protein, 112 aa, synthetic construct
DVLMTQTPLSLPVSLGDQASISCRSSQSIVHTNGNTYLEWYLQNPGQSPKLLIYKVFNRFSGVPDRFSGSGSGTDFTLKISRVEAEDLGVYYCFQGSLFPYTFGGGTKLEIK

SEQ ID NO: 67 - protein, 5 aa, synthetic construct
DYNMH

SEQ ID NO: 68 - protein, 17 aa, synthetic construct
YINPNNGGTTYNQKFKG

SEQ ID NO: 69 - protein, 11 aa, synthetic construct
RGYGSGYAMDY

SEQ ID NO: 70 - protein, 16 aa, synthetic construct
TSSQSIVHTNGNTYLE

SEQ ID NO: 71 - protein, 7 aa, synthetic construct
KVSNRFS

SEQ ID NO: 72 - protein, 9 aa, synthetic construct
FQGSLFPYT

SEQ ID NO: 73 - protein, 120 aa, synthetic construct
EVQLQQSGPELVKPGASVKMSCKASEYTFTDYNMHWVKQSHGKSLEWIGYINPNNGGTTYNQKFKGKATLTVNKSSSTAYMELRSLTSDDSAVYYCARRGYGSGYAMDYWGQGASVTVSS

SEQ ID NO: 74 - protein, 112 aa, synthetic construct
DVLLTQTPLSLPVSLGDRASISCTSSQSIVHTNGNTYLEWYLQNPGQSPKLLIYKVSNRFSGVPDRFSGSGSGTDFTLKISRVEAEDLGVYYCFQGSLFPYTFGGGTKLEIK

SEQ ID NO: 75 - protein, 5 aa, synthetic construct
DYNIH

SEQ ID NO: 76 - protein, 17 aa, synthetic construct
YINPNNGNTNYNQKFEG

SEQ ID NO: 77 - protein, 11 aa, synthetic construct
RGYGSSYAMDF

SEQ ID NO: 78 - protein, 16 aa, synthetic construct
RSSHIIVHTNGNTYLE

SEQ ID NO: 79 - protein, 7 aa, synthetic construct
KVSNRFS

SEQ ID NO: 80 - protein, 9 aa, synthetic construct
FQGSRVPYT

SEQ ID NO: 81 - protein, 120 aa, synthetic construct
EVQLQQSGPELVKPGASLKLSCKASGYTFPDYNIHWVKQSHGKSLEWIGYINPNNGNTNYNQKFEGKATLTVSKSSSTAYMELRSLTSDDSAVYSCARRGYGSSYAMDFWGQGTSVTVSS

SEQ ID NO: 82 - protein, 112 aa, synthetic construct
DVLMTQTPLSLPVSLGNQASISCRSSHIIVHTNGNTYLEWYLQKPGQSPKLLIYKVSNRFSGVPDRFSGSGSGTDFTLKISRVEAEDLGVYYCFQGSRVPYTFGGGTKLEIK

SEQ ID NO: 83 - protein, 17 aa, synthetic construct
YINPNHDATSYNQKFQG

SEQ ID NO: 84 - protein, 16 aa, synthetic construct
RSSHNIVHTNANTYLE

SEQ ID NO: 85 - protein, 17 aa, synthetic construct
TISDAGSYTYYPDNEKG

SEQ ID NO: 86 - protein, 385 aa, synthetic construct
QETELSVSAELVPTSSWNISSELNKDSYLTLDEPMNNITTSLGQTAELHCKVSGNPPPTIRWFKNDAPVVQEPRRLSFRSTIYGSRLRIRNLDTTDTGYFQCVATNGKEVVSSTGVLFVKFGPPPTASPGYSDEYEEDGFCQPYRGIACARFIGNRTVYMESLHMQGEIENQITAAFTMIGTSSHLSDKCSQFAIPSLCHYAFPYCDETSSVPKPRDLCRDECEILENVLCQTEYIFARSNPMILMRLKLPNCEDLPQPESPEAANCIRIGIPMADPINKNHKCYNSTGVDYRGTVSVTKSGRQCQPWNSQYPHTHTFTALRFPELNGGHSYCRNPGNQKEAPWCFTLDENFKSDLCDIPACDSKDSKEKNKMEAHHHHHHHHHH

SEQ ID NO: 87 - protein, 116 aa, synthetic construct
QVQLQESGPGLVKPSQTLSLTCTVSGYAFTAYNIHWVRQAPGQGLEWMGSFDPYDGGSSYNQKFKDRLTISKDTSKNQVVLTMTNMDPVDTATYYCARGWYYFDYWGHGTLVTVSS

SEQ ID NO: 88 - protein, 107 aa, synthetic construct
DIVMTQTPLSLPVTPGEPASISCRASKSISKYLAWYQQKPGQAPRLLIYSGSTLQSGIPPRFSGSGYGTDFTLTINNIESEDAAYYFCQQHDESPYTFGEGTKVEIK

SEQ ID NO: 89 - protein, 472 aa, synthetic construct
MHRPRRRGTRPPLLALLAALLLAARGAAAQETELSVSAELVPTSSWNISSELNKDSYLTLDEPMNNITTSLGQTAELHCKVSGNPPPTIRWFKNDAPVVQEPRRLSFRSTIYGSRLRIRNLDTTDTGYFQCVATNGKEVVSSTGVLFVKFGPPPTASPGYSDEYEEDGFCQPYRGIACARFIGNRTVYMESLHMQGEIENQITAAFTMIGTSSHLSDKCSQFAIPSLCHYAFPYCDETSSVPKPRDLCRDECEILENVLCQTEYIFARSNPMILMRLKLPNCEDLPQPESPEAANCIRIGIPMADPINKNHKCYNSTGVDYRGTVSVTKSGRQCQPWNSQYPHTHTFTALRFPELNGGHSYCRNPGNQKEAPWCFTLDENFKSDLCDIPACDSKDSKEKNKMEILYILVPSVAIPLAIALLFFFICVCRNNQKSSSAPVQRQPKHVRGQNVEMSMLNAYKPKSKAKELPLSA

SEQ ID NO: 90 - protein, 403 aa, synthetic construct
MHRPRRRGTRPPLLALLAALLLAARGAAAQETELSVSAELVPTSSWNISSELNKDSYLTLDEPMNNITTVVSSTGVLFVKFGPPPTASPGYSDEYEEDGFCQPYRGIACARFIGNRTVYMESLHMQGEIENQITAAFTMIGTSSHLSDKCSQFAIPSLCHYAFPYCDETSSVPKPRDLCRDECEILENVLCQTEYIFARSNPMILMRLKLPNCEDLPQPESPEAANCIRIGIPMADPINKNHKCYNSTGVDYRGTVSVTKSGRQCQPWNSQYPHTHTFTALRFPELNGGHSYCRNPGNQKEAPWCFTLDENFKSDLCDIPACDSKDSKEKNKMEILYILVPSVAIPLAIALLFFFICVCRNNQKSSSAPVQRQPKHVRGQNVEMSMLNAYKPKSKAKELPLSA

SEQ ID NO: 91 - protein, 339 aa, synthetic construct
MHRPRRRGTRPPLLALLAALLLAARGAAAQETELSVSAELVPTSSWNISSELNKDSYLTLDEPMNNITTSLGQTAELHCKVSGNPPPTIRWFKNDAPVVQEPRRLSFRSTIYGSRLRIRNLDTTDTGYFQCVATNGKEVVSSTGVLFVKFGPPPTASPGYSDEYEEDGPMADPINKNHKCYNSTGVDYRGTVSVTKSGRQCQPWNSQYPHTHTFTALRFPELNGGHSYCRNPGNQKEAPWCFTLDENFKSDLCDIPACDSKDSKEKNKMEILYILVPSVAIPLAIALLFFFICVCRNNQKSSSAPVQRQPKHVRGQNVEMSMLNAYKPKSKAKELPLSA

SEQ ID NO: 92 - protein, 389 aa, synthetic construct
MHRPRRRGTRPPLLALLAALLLAARGAAAQETELSVSAELVPTSSWNISSELNKDSYLTLDEPMNNITTSLGQTAELHCKVSGNPPPTIRWFKNDAPVVQEPRRLSFRSTIYGSRLRIRNLDTTDTGYFQCVATNGKEVVSSTGVLFVKFGPPPTASPGYSDEYEEDGFCQPYRGIACARFIGNRTVYMESLHMQGEIENQITAAFTMIGTSSHLSDKCSQFAIPSLCHYAFPYCDETSSVPKPRDLCRDECEILENVLCQTEYIFARSNPMILMRLKLPNCEDLPQPESPEAANCIRIGIPMADPINKNKDSKEKNKMEILYILVPSVAIPLAIALLFFFICVCRNNQKSSSAPVQRQPKHVRGQNVEMSMLNAYKPKSKAKELPLSA

SEQ ID NO: 93 - protein, 121 aa, synthetic construct
EVQLVESGGGLVKPGGSLRLSCAASGFTFNSYAMSWVRQTPEKRLEWVATISDAGSYTYYPDNEKGRFTISRDNAKNNLYLQMNSLRAEDTAIYYCVRGGYYYNLYAMDYWGQGTLVTVSS

SEQ ID NO: 94 - protein, 121 aa, synthetic construct
EVQLVESGGGLVKPGGSLRLSCAASGFTFNSYAMSWVRQTPEKGLEWVATISDAGSYTYYPDNEKGRFTISRDNAKNNLYLQMNSLRAEDTAIYYCVRGGYYYNLYAMDYWGQGTLVTVSS

SEQ ID NO: 95 - protein, 121 aa, synthetic construct
EVQLVESGGGLVKPGGSLRLSCAASGFTFNSYAMSWVRQTPGKRLEWVATISDAGSYTYYPDNEKGRFTISRDNAKNNLYLQMNSLRAEDTAIYYCVRGGYYYNLYAMDYWGQGTLVTVSS

SEQ ID NO: 96 - protein, 121 aa, synthetic construct
EVQLVESGGGLVKPGGSLRLSCAASGFTFNSYAMSWVRQTPEKRLEWVATISDAGSYTYYPDNEKGRFTISRDNAKNSLYLQMNSLRAEDTAIYYCVRGGYYYNLYAMDYWGQGTLVTVSS

SEQ ID NO: 97 - protein, 121 aa, synthetic construct
EVQLVESGGGLVKPGGSLRLSCAASGFTFNSYAMSWVRQTPGKGLEWVATISDAGSYTYYPDNEKGRFTISRDNAKNNLYLQMNSLRAEDTAIYYCVRGGYYYNLYAMDYWGQGTLVTVSS

SEQ ID NO: 98 - protein, 121 aa, synthetic construct
EVQLVESGGGLVKPGGSLRLSCAASGFTFNSYAMSWVRQTPGKGLEWVATISDAGSYTYYPDNEKGRFTISRDNAKNSLYLQMNSLRAEDTAIYYCVRGGYYYNLYAMDYWGQGTLVTVSS

SEQ ID NO: 99 - protein, 121 aa, synthetic construct
EVQLVESGGGLVKPGGSLRLSCAASGFTFNSYAMSWVRQTPEKGLEWVATISDAGSYTYYPDNEKGRFTISRDNAKNSLYLQMNSLRAEDTAIYYCVRGGYYYNLYAMDYWGQGTLVTVSS

SEQ ID NO: 100 - protein, 121 aa, synthetic construct
EVQLVESGGGLVKPGGSLRLSCAASGFTFNSYAMSWVRQTPGKRLEWVATISDAGSYTYYPDNEKGRFTISRDNAKNSLYLQMNSLRAEDTAIYYCVRGGYYYNLYAMDYWGQGTLVTVSS

SEQ ID NO: 101 - protein, 111 aa, synthetic construct
DIVLTQSPDSLAVSLGERATINCKASQSVSFPGTSLMHWYQQKPGQQPKLLIYRASNLEAGVPDRFSGSGSRTDFTLTISSLQAEDVAVYYCQQSREYPWTFGGGTKVEIK